European Patent Specification EP 3 740 483 B1, published January 11, 2023. Title: DNA-PK INHIBITORS. Applicant: Vertex Pharmaceuticals Incorporated MAHAJAN, Sudipta WEINBERG, Marc Saul D'ASTOLFO, Diego Sebastian. The sequence listing filed with the application follows.

SEQUENCE LISTING (12 sequences)

SEQ ID NO: 1 - DNA, 20 bp, Artificial Sequence
  AAVS1 target site
accccacagtggggccacta

SEQ ID NO: 2 - DNA, 20 bp, Artificial Sequence
  NAV1.7 target
ggctgagcgtccatcaacca

SEQ ID NO: 3 - RNA, 100 nt, Artificial Sequence
  AAVS1 sgRNA
  misc_feature (1)..(3): 2'-O-methyl 3'-phosphorothioate
  misc_feature (97)..(99): 2'-O-methyl 3'-phosphorothioate
accccacaguggggccacuaguuuuagagcuagaaauagcaaguuaaaauaaggcuaguccguuaucaacuugaaaaaguggcaccgagucggugcuuuu

SEQ ID NO: 4 - RNA, 100 nt, Artificial Sequence
  NAV1.7 sgRNA
  misc_feature (1)..(3): 2'-O-methyl 3'-phosphorothioate
  misc_feature (97)..(99): 2'-O-methyl 3'-phosphorothioate
ggcugagcguccaucaaccaguuuuagagcuagaaauagcaaguuaaaauaaggcuaguccguuaucaacuugaaaaaguggcaccgagucggugcuuuu

SEQ ID NO: 5 - DNA, 90 bp, Artificial Sequence
  AAVS1 PAM
  misc_feature (1)..(3): 2'-O-methyl 3'-phosphorothioate
  misc_feature (87)..(89): 2'-O-methyl 3'-phosphorothioate
gggtacttttatctgtcccctccaccccacagtggggccagaattctcagctagggacaggattggtgacagaaaagccccatccttagg

SEQ ID NO: 6 - DNA, 90 bp, Artificial Sequence
  AAVS1 Non-PAM
  misc_feature (1)..(3): 2'-O-methyl 3'-phosphorothioate
  misc_feature (87)..(89): 2'-O-methyl 3'-phosphorothioate
cctaaggatggggcttttctgtcaccaatcctgtccctagctgagaattctggccccactgtggggtggaggggacagataaaagtaccc

SEQ ID NO: 7 - DNA, 90 bp, Artificial Sequence
  NAV1.7 PAM
  misc_feature (1)..(3): 2'-O-methyl 3'-phosphorothioate
  misc_feature (87)..(89): 2'-O-methyl 3'-phosphorothioate
agctgtccattggggagcatgagggctgagcgtccatcaactgagaattcccagggagaccacaccgttgcagtccacagcactgtgcat

SEQ ID NO: 8 - DNA, 90 bp, Artificial Sequence
  NAV1.7 Non-PAM
  misc_feature (1)..(3): 2'-O-methyl 3'-phosphorothioate
  misc_feature (87)..(89): 2'-O-methyl 3'-phosphorothioate
atgcacagtgctgtggactgcaacggtgtggtctccctgggaattctcagttgatggacgctcagccctcatgctccccaatggacagct

SEQ ID NO: 9 - DNA, 20 bp, Artificial Sequence
  AAVS1 FW
ggacaaccccaaagtacccc

SEQ ID NO: 10 - DNA, 20 bp, Artificial Sequence
  AAVS1 RV
aggatcagtgaaacgcacca

SEQ ID NO: 11 - DNA, 20 bp, Artificial Sequence
  NAV1.7 FW
gccagtgggttcagtggtat

SEQ ID NO: 12 - DNA, 25 bp, Artificial Sequence
  NAV1.7 RV
tcagcattatccttgcattttctgt